European Patent Application EP 4 772 631 A1, published July 8, 2026. Title: 抑制C3基因表达的双链寡核苷酸、缀合物以及它们的用途. Applicant: 苏州炫景生物科技有限公司. The sequence listing filed with the application follows.

SEQUENCE LISTING (424 sequences)

SEQ ID NO: 1 - RNA, 19 nt, synthetic construct
  source 1..19: mol_type = other RNA
gtccacgacttcccaggca

SEQ ID NO: 2 - RNA, 19 nt, synthetic construct
  source 1..19: mol_type = other RNA
ccacgacttcccaggcaaa

SEQ ID NO: 3 - RNA, 19 nt, synthetic construct
  source 1..19: mol_type = other RNA
cacgacttcccaggcaaaa

SEQ ID NO: 4 - RNA, 19 nt, synthetic construct
  source 1..19: mol_type = other RNA
gtgctgtccagtgagaaga

SEQ ID NO: 5 - RNA, 19 nt, synthetic construct
  source 1..19: mol_type = other RNA
gctgtccagtgagaagact

SEQ ID NO: 6 - RNA, 19 nt, synthetic construct
  source 1..19: mol_type = other RNA
cagagcgggtacctcttca

SEQ ID NO: 7 - RNA, 19 nt, synthetic construct
  source 1..19: mol_type = other RNA
gcgggtacctcttcatcca

SEQ ID NO: 8 - RNA, 19 nt, synthetic construct
  source 1..19: mol_type = other RNA
cagacagacaagaccatct

SEQ ID NO: 9 - RNA, 19 nt, synthetic construct
  source 1..19: mol_type = other RNA
ggatcttcaccgtcaacca

SEQ ID NO: 10 - RNA, 19 nt, synthetic construct
  source 1..19: mol_type = other RNA
ccgtcaaccacaagctgct

SEQ ID NO: 11 - RNA, 19 nt, synthetic construct
  source 1..19: mol_type = other RNA
cgtcaaccacaagctgcta

SEQ ID NO: 12 - RNA, 19 nt, synthetic construct
  source 1..19: mol_type = other RNA
cggtcaagcaggactcctt

SEQ ID NO: 13 - RNA, 19 nt, synthetic construct
  source 1..19: mol_type = other RNA
gtcaagcaggactccttgt

SEQ ID NO: 14 - RNA, 19 nt, synthetic construct
  source 1..19: mol_type = other RNA
caagcaggactccttgtct

SEQ ID NO: 15 - RNA, 19 nt, synthetic construct
  source 1..19: mol_type = other RNA
cttgggacattccggaact

SEQ ID NO: 16 - RNA, 19 nt, synthetic construct
  source 1..19: mol_type = other RNA
gggacattccggaactcgt

SEQ ID NO: 17 - RNA, 19 nt, synthetic construct
  source 1..19: mol_type = other RNA
cagtggaagatccgagcct

SEQ ID NO: 18 - RNA, 19 nt, synthetic construct
  source 1..19: mol_type = other RNA
agtggaagatccgagccta

SEQ ID NO: 19 - RNA, 19 nt, synthetic construct
  source 1..19: mol_type = other RNA
ggaagatccgagcctacta

SEQ ID NO: 20 - RNA, 19 nt, synthetic construct
  source 1..19: mol_type = other RNA
gaagatccgagcctactat

SEQ ID NO: 21 - RNA, 19 nt, synthetic construct
  source 1..19: mol_type = other RNA
gatccgagcctactatgaa

SEQ ID NO: 22 - RNA, 19 nt, synthetic construct
  source 1..19: mol_type = other RNA
agtttgaggtgaaggagta

SEQ ID NO: 23 - RNA, 19 nt, synthetic construct
  source 1..19: mol_type = other RNA
gcccagtttcgaggtcata

SEQ ID NO: 24 - RNA, 19 nt, synthetic construct
  source 1..19: mol_type = other RNA
ccagtttcgaggtcatagt

SEQ ID NO: 25 - RNA, 19 nt, synthetic construct
  source 1..19: mol_type = other RNA
cagtttcgaggtcatagtg

SEQ ID NO: 26 - RNA, 19 nt, synthetic construct
  source 1..19: mol_type = other RNA
gtttcgaggtcatagtgga

SEQ ID NO: 27 - RNA, 19 nt, synthetic construct
  source 1..19: mol_type = other RNA
cgaggtcatagtggagcct

SEQ ID NO: 28 - RNA, 19 nt, synthetic construct
  source 1..19: mol_type = other RNA
agtggagcctacagagaaa

SEQ ID NO: 29 - RNA, 19 nt, synthetic construct
  source 1..19: mol_type = other RNA
cagagaaattctactacat

SEQ ID NO: 30 - RNA, 19 nt, synthetic construct
  source 1..19: mol_type = other RNA
aaattctactacatctata

SEQ ID NO: 31 - RNA, 19 nt, synthetic construct
  source 1..19: mol_type = other RNA
ggaactgcctttgtcatct

SEQ ID NO: 32 - RNA, 19 nt, synthetic construct
  source 1..19: mol_type = other RNA
gaactgcctttgtcatctt

SEQ ID NO: 33 - RNA, 19 nt, synthetic construct
  source 1..19: mol_type = other RNA
cctttgtcatcttcgggat

SEQ ID NO: 34 - RNA, 19 nt, synthetic construct
  source 1..19: mol_type = other RNA
ctgaatccctcaagcgcat

SEQ ID NO: 35 - RNA, 19 nt, synthetic construct
  source 1..19: mol_type = other RNA
caggcagtgacatggtgca

SEQ ID NO: 36 - RNA, 19 nt, synthetic construct
  source 1..19: mol_type = other RNA
gtgacctctccctaccaga

SEQ ID NO: 37 - RNA, 19 nt, synthetic construct
  source 1..19: mol_type = other RNA
gaatgccctttgacctcat

SEQ ID NO: 38 - RNA, 19 nt, synthetic construct
  source 1..19: mol_type = other RNA
cctttgacctcatggtgtt

SEQ ID NO: 39 - RNA, 19 nt, synthetic construct
  source 1..19: mol_type = other RNA
gacctcatggtgttcgtga

SEQ ID NO: 40 - RNA, 19 nt, synthetic construct
  source 1..19: mol_type = other RNA
ctcatggtgttcgtgacga

SEQ ID NO: 41 - RNA, 19 nt, synthetic construct
  source 1..19: mol_type = other RNA
tcatggtgttcgtgacgaa

SEQ ID NO: 42 - RNA, 19 nt, synthetic construct
  source 1..19: mol_type = other RNA
ctgtgcagtctctaaccca

SEQ ID NO: 43 - RNA, 19 nt, synthetic construct
  source 1..19: mol_type = other RNA
gccagaagcccttgagcat

SEQ ID NO: 44 - RNA, 19 nt, synthetic construct
  source 1..19: mol_type = other RNA
cagaagcccttgagcatca

SEQ ID NO: 45 - RNA, 19 nt, synthetic construct
  source 1..19: mol_type = other RNA
gcatcacggtgcgcacgaa

SEQ ID NO: 46 - RNA, 19 nt, synthetic construct
  source 1..19: mol_type = other RNA
cggtgcgcacgaagaagca

SEQ ID NO: 47 - RNA, 19 nt, synthetic construct
  source 1..19: mol_type = other RNA
ccgtgggcaactccaacaa

SEQ ID NO: 48 - RNA, 19 nt, synthetic construct
  source 1..19: mol_type = other RNA
cgtgggcaactccaacaat

SEQ ID NO: 49 - RNA, 19 nt, synthetic construct
  source 1..19: mol_type = other RNA
gtgggcaactccaacaatt

SEQ ID NO: 50 - RNA, 19 nt, synthetic construct
  source 1..19: mol_type = other RNA
gcaactccaacaattacct

SEQ ID NO: 51 - RNA, 19 nt, synthetic construct
  source 1..19: mol_type = other RNA
ctccaacaattacctgcat

SEQ ID NO: 52 - RNA, 19 nt, synthetic construct
  source 1..19: mol_type = other RNA
ggggagaccctcaacgtca

SEQ ID NO: 53 - RNA, 19 nt, synthetic construct
  source 1..19: mol_type = other RNA
gggagaccctcaacgtcaa

SEQ ID NO: 54 - RNA, 19 nt, synthetic construct
  source 1..19: mol_type = other RNA
gagaccctcaacgtcaact

SEQ ID NO: 55 - RNA, 19 nt, synthetic construct
  source 1..19: mol_type = other RNA
ccctcaacgtcaacttcct

SEQ ID NO: 56 - RNA, 19 nt, synthetic construct
  source 1..19: mol_type = other RNA
tcaacttcctcctgcgaat

SEQ ID NO: 57 - RNA, 19 nt, synthetic construct
  source 1..19: mol_type = other RNA
gaggccaagatccgctact

SEQ ID NO: 58 - RNA, 19 nt, synthetic construct
  source 1..19: mol_type = other RNA
agatccgctactacaccta

SEQ ID NO: 59 - RNA, 19 nt, synthetic construct
  source 1..19: mol_type = other RNA
cgctactacacctacctga

SEQ ID NO: 60 - RNA, 19 nt, synthetic construct
  source 1..19: mol_type = other RNA
gctactacacctacctgat

SEQ ID NO: 61 - RNA, 19 nt, synthetic construct
  source 1..19: mol_type = other RNA
ccgtgtgggtggacgtcaa

SEQ ID NO: 62 - RNA, 19 nt, synthetic construct
  source 1..19: mol_type = other RNA
gggctcgctggtggtaaaa

SEQ ID NO: 63 - RNA, 19 nt, synthetic construct
  source 1..19: mol_type = other RNA
ccctgaagatagagggtga

SEQ ID NO: 64 - RNA, 19 nt, synthetic construct
  source 1..19: mol_type = other RNA
cgggagaaccccatgaggt

SEQ ID NO: 65 - RNA, 19 nt, synthetic construct
  source 1..19: mol_type = other RNA
gggagaaccccatgaggtt

SEQ ID NO: 66 - RNA, 19 nt, synthetic construct
  source 1..19: mol_type = other RNA
gagaaccccatgaggttct

SEQ ID NO: 67 - RNA, 19 nt, synthetic construct
  source 1..19: mol_type = other RNA
ctgctgcaactacatcaca

SEQ ID NO: 68 - RNA, 19 nt, synthetic construct
  source 1..19: mol_type = other RNA
ggagtaacctggatgagga

SEQ ID NO: 69 - RNA, 19 nt, synthetic construct
  source 1..19: mol_type = other RNA
gtaacctggatgaggacat

SEQ ID NO: 70 - RNA, 19 nt, synthetic construct
  source 1..19: mol_type = other RNA
gcagaagagaacatcgttt

SEQ ID NO: 71 - RNA, 19 nt, synthetic construct
  source 1..19: mol_type = other RNA
gagaacatcgtttcccgaa

SEQ ID NO: 72 - RNA, 19 nt, synthetic construct
  source 1..19: mol_type = other RNA
cccgaagtgagttcccaga

SEQ ID NO: 73 - RNA, 19 nt, synthetic construct
  source 1..19: mol_type = other RNA
cgaagctcatgaatatatt

SEQ ID NO: 74 - RNA, 19 nt, synthetic construct
  source 1..19: mol_type = other RNA
gaagctcatgaatatattt

SEQ ID NO: 75 - RNA, 19 nt, synthetic construct
  source 1..19: mol_type = other RNA
cccttcgaggtcacagtaa

SEQ ID NO: 76 - RNA, 19 nt, synthetic construct
  source 1..19: mol_type = other RNA
ccttcgaggtcacagtaat

SEQ ID NO: 77 - RNA, 19 nt, synthetic construct
  source 1..19: mol_type = other RNA
tcacagtaatgcaggactt

SEQ ID NO: 78 - RNA, 19 nt, synthetic construct
  source 1..19: mol_type = other RNA
cctgcggctaccctactct

SEQ ID NO: 79 - RNA, 19 nt, synthetic construct
  source 1..19: mol_type = other RNA
gcggctaccctactctgtt

SEQ ID NO: 80 - RNA, 19 nt, synthetic construct
  source 1..19: mol_type = other RNA
ggctaccctactctgttgt

SEQ ID NO: 81 - RNA, 19 nt, synthetic construct
  source 1..19: mol_type = other RNA
gctaccctactctgttgtt

SEQ ID NO: 82 - RNA, 19 nt, synthetic construct
  source 1..19: mol_type = other RNA
accctactctgttgttcga

SEQ ID NO: 83 - RNA, 19 nt, synthetic construct
  source 1..19: mol_type = other RNA
ccctactctgttgttcgaa

SEQ ID NO: 84 - RNA, 19 nt, synthetic construct
  source 1..19: mol_type = other RNA
cctactctgttgttcgaaa

SEQ ID NO: 85 - RNA, 19 nt, synthetic construct
  source 1..19: mol_type = other RNA
cgaaacgagcaggtggaaa

SEQ ID NO: 86 - RNA, 19 nt, synthetic construct
  source 1..19: mol_type = other RNA
gaaacgagcaggtggaaat

SEQ ID NO: 87 - RNA, 19 nt, synthetic construct
  source 1..19: mol_type = other RNA
cgagcaggtggaaatccga

SEQ ID NO: 88 - RNA, 19 nt, synthetic construct
  source 1..19: mol_type = other RNA
caattaccggcagaaccaa

SEQ ID NO: 89 - RNA, 19 nt, synthetic construct
  source 1..19: mol_type = other RNA
gggtggaactactccacaa

SEQ ID NO: 90 - RNA, 19 nt, synthetic construct
  source 1..19: mol_type = other RNA
ggtggaactactccacaat

SEQ ID NO: 91 - RNA, 19 nt, synthetic construct
  source 1..19: mol_type = other RNA
ggaactactccacaatcca

SEQ ID NO: 92 - RNA, 19 nt, synthetic construct
  source 1..19: mol_type = other RNA
cgtcaccagcagaccgtaa

SEQ ID NO: 93 - RNA, 19 nt, synthetic construct
  source 1..19: mol_type = other RNA
caccagcagaccgtaacca

SEQ ID NO: 94 - RNA, 19 nt, synthetic construct
  source 1..19: mol_type = other RNA
ggaagtccctgaaggtcgt

SEQ ID NO: 95 - RNA, 19 nt, synthetic construct
  source 1..19: mol_type = other RNA
gtcgtgccggaaggaatca

SEQ ID NO: 96 - RNA, 19 nt, synthetic construct
  source 1..19: mol_type = other RNA
cgtgccggaaggaatcaga

SEQ ID NO: 97 - RNA, 19 nt, synthetic construct
  source 1..19: mol_type = other RNA
gtgccggaaggaatcagaa

SEQ ID NO: 98 - RNA, 19 nt, synthetic construct
  source 1..19: mol_type = other RNA
ccggaaggaatcagaatga

SEQ ID NO: 99 - RNA, 19 nt, synthetic construct
  source 1..19: mol_type = other RNA
cggaaggaatcagaatgaa

SEQ ID NO: 100 - RNA, 19 nt, synthetic construct
  source 1..19: mol_type = other RNA
tgcagacctcagtgaccaa

SEQ ID NO: 101 - RNA, 19 nt, synthetic construct
  source 1..19: mol_type = other RNA
gaccagaattctcctgcaa

SEQ ID NO: 102 - RNA, 19 nt, synthetic construct
  source 1..19: mol_type = other RNA
gaacggctgaagcacctca

SEQ ID NO: 103 - RNA, 19 nt, synthetic construct
  source 1..19: mol_type = other RNA
cgctgtgcattacctggat

SEQ ID NO: 104 - RNA, 19 nt, synthetic construct
  source 1..19: mol_type = other RNA
gcattacctggatgaaacg

SEQ ID NO: 105 - RNA, 19 nt, synthetic construct
  source 1..19: mol_type = other RNA
ccttggagctcatcaagaa

SEQ ID NO: 106 - RNA, 19 nt, synthetic construct
  source 1..19: mol_type = other RNA
gcagctggccttcagacaa

SEQ ID NO: 107 - RNA, 19 nt, synthetic construct
  source 1..19: mol_type = other RNA
ccgcctacgtggtcaaggt

SEQ ID NO: 108 - RNA, 19 nt, synthetic construct
  source 1..19: mol_type = other RNA
cctacgtggtcaaggtctt

SEQ ID NO: 109 - RNA, 19 nt, synthetic construct
  source 1..19: mol_type = other RNA
cgtggtcaaggtcttctct

SEQ ID NO: 110 - RNA, 19 nt, synthetic construct
  source 1..19: mol_type = other RNA
ctctggctgtcaacctcat

SEQ ID NO: 111 - RNA, 19 nt, synthetic construct
  source 1..19: mol_type = other RNA
ctctgcggggctgttaaat

SEQ ID NO: 112 - RNA, 19 nt, synthetic construct
  source 1..19: mol_type = other RNA
ctgttaaatggctgatcct

SEQ ID NO: 113 - RNA, 19 nt, synthetic construct
  source 1..19: mol_type = other RNA
ggaggatgcgcccgtgata

SEQ ID NO: 114 - RNA, 19 nt, synthetic construct
  source 1..19: mol_type = other RNA
ggccctcacggcctttgtt

SEQ ID NO: 115 - RNA, 19 nt, synthetic construct
  source 1..19: mol_type = other RNA
ctcacggcctttgttctca

SEQ ID NO: 116 - RNA, 19 nt, synthetic construct
  source 1..19: mol_type = other RNA
cctttgttctcatctcgct

SEQ ID NO: 117 - RNA, 19 nt, synthetic construct
  source 1..19: mol_type = other RNA
cttgaagccaactacatga

SEQ ID NO: 118 - RNA, 19 nt, synthetic construct
  source 1..19: mol_type = other RNA
ccaactacatgaacctaca

SEQ ID NO: 119 - RNA, 19 nt, synthetic construct
  source 1..19: mol_type = other RNA
cctacagagatcctacact

SEQ ID NO: 120 - RNA, 19 nt, synthetic construct
  source 1..19: mol_type = other RNA
ctgaccacagccaaagata

SEQ ID NO: 121 - RNA, 19 nt, synthetic construct
  source 1..19: mol_type = other RNA
ccacagccaaagataagaa

SEQ ID NO: 122 - RNA, 19 nt, synthetic construct
  source 1..19: mol_type = other RNA
gccaaagataagaaccgct

SEQ ID NO: 123 - RNA, 19 nt, synthetic construct
  source 1..19: mol_type = other RNA
gccacatcctatgccctct

SEQ ID NO: 124 - RNA, 19 nt, synthetic construct
  source 1..19: mol_type = other RNA
ccacatcctatgccctctt

SEQ ID NO: 125 - RNA, 19 nt, synthetic construct
  source 1..19: mol_type = other RNA
ggccctactgcagctaaaa

SEQ ID NO: 126 - RNA, 19 nt, synthetic construct
  source 1..19: mol_type = other RNA
ctactgcagctaaaagact

SEQ ID NO: 127 - RNA, 19 nt, synthetic construct
  source 1..19: mol_type = other RNA
cagctaaaagactttgact

SEQ ID NO: 128 - RNA, 19 nt, synthetic construct
  source 1..19: mol_type = other RNA
gctaaaagactttgacttt

SEQ ID NO: 129 - RNA, 19 nt, synthetic construct
  source 1..19: mol_type = other RNA
ccgtcgtgcgttggctcaa

SEQ ID NO: 130 - RNA, 19 nt, synthetic construct
  source 1..19: mol_type = other RNA
cgtcgtgcgttggctcaat

SEQ ID NO: 131 - RNA, 19 nt, synthetic construct
  source 1..19: mol_type = other RNA
cgtgcgttggctcaatgaa

SEQ ID NO: 132 - RNA, 19 nt, synthetic construct
  source 1..19: mol_type = other RNA
cgttggctcaatgaacaga

SEQ ID NO: 133 - RNA, 19 nt, synthetic construct
  source 1..19: mol_type = other RNA
ggctcaatgaacagagata

SEQ ID NO: 134 - RNA, 19 nt, synthetic construct
  source 1..19: mol_type = other RNA
ctcaatgaacagagatact

SEQ ID NO: 135 - RNA, 19 nt, synthetic construct
  source 1..19: mol_type = other RNA
ccaccttcatggtgttcca

SEQ ID NO: 136 - RNA, 19 nt, synthetic construct
  source 1..19: mol_type = other RNA
caccttcatggtgttccaa

SEQ ID NO: 137 - RNA, 19 nt, synthetic construct
  source 1..19: mol_type = other RNA
ggtgttccaagccttggct

SEQ ID NO: 138 - RNA, 19 nt, synthetic construct
  source 1..19: mol_type = other RNA
ccgtatccactgggaatct

SEQ ID NO: 139 - RNA, 19 nt, synthetic construct
  source 1..19: mol_type = other RNA
gcctcctgcgatcagaaga

SEQ ID NO: 140 - RNA, 19 nt, synthetic construct
  source 1..19: mol_type = other RNA
tgcgatcagaagagaccaa

SEQ ID NO: 141 - RNA, 19 nt, synthetic construct
  source 1..19: mol_type = other RNA
gatcagaagagaccaagga

SEQ ID NO: 142 - RNA, 19 nt, synthetic construct
  source 1..19: mol_type = other RNA
gtttcacagtcacagctga

SEQ ID NO: 143 - RNA, 19 nt, synthetic construct
  source 1..19: mol_type = other RNA
tgacaatgtaccatgctaa

SEQ ID NO: 144 - RNA, 19 nt, synthetic construct
  source 1..19: mol_type = other RNA
gtaccatgctaaggccaaa

SEQ ID NO: 145 - RNA, 19 nt, synthetic construct
  source 1..19: mol_type = other RNA
caactcacctgtaataaat

SEQ ID NO: 146 - RNA, 19 nt, synthetic construct
  source 1..19: mol_type = other RNA
cctgtaataaattcgacct

SEQ ID NO: 147 - RNA, 19 nt, synthetic construct
  source 1..19: mol_type = other RNA
gtaataaattcgacctcaa

SEQ ID NO: 148 - RNA, 19 nt, synthetic construct
  source 1..19: mol_type = other RNA
cgacctcaaggtcaccata

SEQ ID NO: 149 - RNA, 19 nt, synthetic construct
  source 1..19: mol_type = other RNA
gacctcaaggtcaccataa

SEQ ID NO: 150 - RNA, 19 nt, synthetic construct
  source 1..19: mol_type = other RNA
caaggtcaccataaaacca

SEQ ID NO: 151 - RNA, 19 nt, synthetic construct
  source 1..19: mol_type = other RNA
ccagcaccggaaacagaaa

SEQ ID NO: 152 - RNA, 19 nt, synthetic construct
  source 1..19: mol_type = other RNA
gcaccggaaacagaaaaga

SEQ ID NO: 153 - RNA, 19 nt, synthetic construct
  source 1..19: mol_type = other RNA
ggcctcaggatgccaagaa

SEQ ID NO: 154 - RNA, 19 nt, synthetic construct
  source 1..19: mol_type = other RNA
caggatgccaagaacacta

SEQ ID NO: 155 - RNA, 19 nt, synthetic construct
  source 1..19: mol_type = other RNA
gatgccaagaacactatga

SEQ ID NO: 156 - RNA, 19 nt, synthetic construct
  source 1..19: mol_type = other RNA
ccaagaacactatgatcct

SEQ ID NO: 157 - RNA, 19 nt, synthetic construct
  source 1..19: mol_type = other RNA
agaacactatgatccttga

SEQ ID NO: 158 - RNA, 19 nt, synthetic construct
  source 1..19: mol_type = other RNA
gagaccaggatgccactat

SEQ ID NO: 159 - RNA, 19 nt, synthetic construct
  source 1..19: mol_type = other RNA
ccaggatgccactatgtct

SEQ ID NO: 160 - RNA, 19 nt, synthetic construct
  source 1..19: mol_type = other RNA
caggatgccactatgtcta

SEQ ID NO: 161 - RNA, 19 nt, synthetic construct
  source 1..19: mol_type = other RNA
ggatgccactatgtctata

SEQ ID NO: 162 - RNA, 19 nt, synthetic construct
  source 1..19: mol_type = other RNA
gatgccactatgtctatat

SEQ ID NO: 163 - RNA, 19 nt, synthetic construct
  source 1..19: mol_type = other RNA
gttgacagatacatctcca

SEQ ID NO: 164 - RNA, 19 nt, synthetic construct
  source 1..19: mol_type = other RNA
gacagatacatctccaagt

SEQ ID NO: 165 - RNA, 19 nt, synthetic construct
  source 1..19: mol_type = other RNA
cagatacatctccaagtat

SEQ ID NO: 166 - RNA, 19 nt, synthetic construct
  source 1..19: mol_type = other RNA
agatacatctccaagtatg

SEQ ID NO: 167 - RNA, 19 nt, synthetic construct
  source 1..19: mol_type = other RNA
gatacatctccaagtatga

SEQ ID NO: 168 - RNA, 19 nt, synthetic construct
  source 1..19: mol_type = other RNA
ccaagtatgagctggacaa

SEQ ID NO: 169 - RNA, 19 nt, synthetic construct
  source 1..19: mol_type = other RNA
ggacaaagccttctccgat

SEQ ID NO: 170 - RNA, 19 nt, synthetic construct
  source 1..19: mol_type = other RNA
gacaaagccttctccgata

SEQ ID NO: 171 - RNA, 19 nt, synthetic construct
  source 1..19: mol_type = other RNA
gccttctccgataggaaca

SEQ ID NO: 172 - RNA, 19 nt, synthetic construct
  source 1..19: mol_type = other RNA
ccgataggaacaccctcat

SEQ ID NO: 173 - RNA, 19 nt, synthetic construct
  source 1..19: mol_type = other RNA
gataggaacaccctcatca

SEQ ID NO: 174 - RNA, 19 nt, synthetic construct
  source 1..19: mol_type = other RNA
ctggacaaggtctcacact

SEQ ID NO: 175 - RNA, 19 nt, synthetic construct
  source 1..19: mol_type = other RNA
gctttcaaagttcaccaat

SEQ ID NO: 176 - RNA, 19 nt, synthetic construct
  source 1..19: mol_type = other RNA
ctttcaaagttcaccaata

SEQ ID NO: 177 - RNA, 19 nt, synthetic construct
  source 1..19: mol_type = other RNA
cagtcaaggtctacgccta

SEQ ID NO: 178 - RNA, 19 nt, synthetic construct
  source 1..19: mol_type = other RNA
gtcaaggtctacgcctatt

SEQ ID NO: 179 - RNA, 19 nt, synthetic construct
  source 1..19: mol_type = other RNA
aggtctacgcctattacaa

SEQ ID NO: 180 - RNA, 19 nt, synthetic construct
  source 1..19: mol_type = other RNA
gctgtacccggttctacca

SEQ ID NO: 181 - RNA, 19 nt, synthetic construct
  source 1..19: mol_type = other RNA
ctgtacccggttctaccat

SEQ ID NO: 182 - RNA, 19 nt, synthetic construct
  source 1..19: mol_type = other RNA
ccggaaaaggaggatggaa

SEQ ID NO: 183 - RNA, 19 nt, synthetic construct
  source 1..19: mol_type = other RNA
cggaaaaggaggatggaaa

SEQ ID NO: 184 - RNA, 19 nt, synthetic construct
  source 1..19: mol_type = other RNA
gaggatggaaagctgaaca

SEQ ID NO: 185 - RNA, 19 nt, synthetic construct
  source 1..19: mol_type = other RNA
gccgctgtgctgaggagaa

SEQ ID NO: 186 - RNA, 19 nt, synthetic construct
  source 1..19: mol_type = other RNA
ccgctgtgctgaggagaat

SEQ ID NO: 187 - RNA, 19 nt, synthetic construct
  source 1..19: mol_type = other RNA
cgctgtgctgaggagaatt

SEQ ID NO: 188 - RNA, 19 nt, synthetic construct
  source 1..19: mol_type = other RNA
gtgctgaggagaattgctt

SEQ ID NO: 189 - RNA, 19 nt, synthetic construct
  source 1..19: mol_type = other RNA
gctgaggagaattgcttca

SEQ ID NO: 190 - RNA, 19 nt, synthetic construct
  source 1..19: mol_type = other RNA
ggagaattgcttcatacaa

SEQ ID NO: 191 - RNA, 19 nt, synthetic construct
  source 1..19: mol_type = other RNA
gagaattgcttcatacaaa

SEQ ID NO: 192 - RNA, 19 nt, synthetic construct
  source 1..19: mol_type = other RNA
gtgagccaggagtggacta

SEQ ID NO: 193 - RNA, 19 nt, synthetic construct
  source 1..19: mol_type = other RNA
ccaggagtggactatgtgt

SEQ ID NO: 194 - RNA, 19 nt, synthetic construct
  source 1..19: mol_type = other RNA
caggagtggactatgtgta

SEQ ID NO: 195 - RNA, 19 nt, synthetic construct
  source 1..19: mol_type = other RNA
ggagtggactatgtgtaca

SEQ ID NO: 196 - RNA, 19 nt, synthetic construct
  source 1..19: mol_type = other RNA
gagtggactatgtgtacaa

SEQ ID NO: 197 - RNA, 19 nt, synthetic construct
  source 1..19: mol_type = other RNA
gtggactatgtgtacaaga

SEQ ID NO: 198 - RNA, 19 nt, synthetic construct
  source 1..19: mol_type = other RNA
ccaatgactttgacgagta

SEQ ID NO: 199 - RNA, 19 nt, synthetic construct
  source 1..19: mol_type = other RNA
gactttgacgagtacatca

SEQ ID NO: 200 - RNA, 19 nt, synthetic construct
  source 1..19: mol_type = other RNA
actttgacgagtacatcat

SEQ ID NO: 201 - RNA, 19 nt, synthetic construct
  source 1..19: mol_type = other RNA
gacgagtacatcatggcca

SEQ ID NO: 202 - RNA, 19 nt, synthetic construct
  source 1..19: mol_type = other RNA
catcaagtcaggctcggat

SEQ ID NO: 203 - RNA, 19 nt, synthetic construct
  source 1..19: mol_type = other RNA
caggctcggatgaggtgca

SEQ ID NO: 204 - RNA, 19 nt, synthetic construct
  source 1..19: mol_type = other RNA
gctcggatgaggtgcaggt

SEQ ID NO: 205 - RNA, 19 nt, synthetic construct
  source 1..19: mol_type = other RNA
cgttcatcagccccatcaa

SEQ ID NO: 206 - RNA, 19 nt, synthetic construct
  source 1..19: mol_type = other RNA
ggggtctctcctccgattt

SEQ ID NO: 207 - RNA, 19 nt, synthetic construct
  source 1..19: mol_type = other RNA
ccgatttctggggagagaa

SEQ ID NO: 208 - RNA, 19 nt, synthetic construct
  source 1..19: mol_type = other RNA
ctcagctacatcatcggga

SEQ ID NO: 209 - RNA, 19 nt, synthetic construct
  source 1..19: mol_type = other RNA
gctacatcatcgggaagga

SEQ ID NO: 210 - RNA, 19 nt, synthetic construct
  source 1..19: mol_type = other RNA
ccgaggaggacgaatgcca

SEQ ID NO: 211 - RNA, 19 nt, synthetic construct
  source 1..19: mol_type = other RNA
cgaggaggacgaatgccaa

SEQ ID NO: 212 - RNA, 19 nt, synthetic construct
  source 1..19: mol_type = other RNA
ctttgggtgccccaactga

SEQ ID NO: 213 - RNA, 21 nt, synthetic construct
  source 1..21: mol_type = other RNA
tgcctgggaagtcgtggacag

SEQ ID NO: 214 - RNA, 21 nt, synthetic construct
  source 1..21: mol_type = other RNA
tttgcctgggaagtcgtggac

SEQ ID NO: 215 - RNA, 21 nt, synthetic construct
  source 1..21: mol_type = other RNA
ttttgcctgggaagtcgtgga

SEQ ID NO: 216 - RNA, 21 nt, synthetic construct
  source 1..21: mol_type = other RNA
tcttctcactggacagcacta

SEQ ID NO: 217 - RNA, 21 nt, synthetic construct
  source 1..21: mol_type = other RNA
agtcttctcactggacagcac

SEQ ID NO: 218 - RNA, 21 nt, synthetic construct
  source 1..21: mol_type = other RNA
tgaagaggtacccgctctgca

SEQ ID NO: 219 - RNA, 21 nt, synthetic construct
  source 1..21: mol_type = other RNA
tggatgaagaggtacccgctc

SEQ ID NO: 220 - RNA, 21 nt, synthetic construct
  source 1..21: mol_type = other RNA
agatggtcttgtctgtctgga

SEQ ID NO: 221 - RNA, 21 nt, synthetic construct
  source 1..21: mol_type = other RNA
tggttgacggtgaagatccga

SEQ ID NO: 222 - RNA, 21 nt, synthetic construct
  source 1..21: mol_type = other RNA
agcagcttgtggttgacggtg

SEQ ID NO: 223 - RNA, 21 nt, synthetic construct
  source 1..21: mol_type = other RNA
tagcagcttgtggttgacggt

SEQ ID NO: 224 - RNA, 21 nt, synthetic construct
  source 1..21: mol_type = other RNA
aaggagtcctgcttgaccggg

SEQ ID NO: 225 - RNA, 21 nt, synthetic construct
  source 1..21: mol_type = other RNA
acaaggagtcctgcttgaccg

SEQ ID NO: 226 - RNA, 21 nt, synthetic construct
  source 1..21: mol_type = other RNA
agacaaggagtcctgcttgac

SEQ ID NO: 227 - RNA, 21 nt, synthetic construct
  source 1..21: mol_type = other RNA
agttccggaatgtcccaagac

SEQ ID NO: 228 - RNA, 21 nt, synthetic construct
  source 1..21: mol_type = other RNA
acgagttccggaatgtcccaa

SEQ ID NO: 229 - RNA, 21 nt, synthetic construct
  source 1..21: mol_type = other RNA
aggctcggatcttccactggc

SEQ ID NO: 230 - RNA, 21 nt, synthetic construct
  source 1..21: mol_type = other RNA
taggctcggatcttccactgg

SEQ ID NO: 231 - RNA, 21 nt, synthetic construct
  source 1..21: mol_type = other RNA
tagtaggctcggatcttccac

SEQ ID NO: 232 - RNA, 21 nt, synthetic construct
  source 1..21: mol_type = other RNA
atagtaggctcggatcttcca

SEQ ID NO: 233 - RNA, 21 nt, synthetic construct
  source 1..21: mol_type = other RNA
ttcatagtaggctcggatctt

SEQ ID NO: 234 - RNA, 21 nt, synthetic construct
  source 1..21: mol_type = other RNA
tactccttcacctcaaactca

SEQ ID NO: 235 - RNA, 21 nt, synthetic construct
  source 1..21: mol_type = other RNA
tatgacctcgaaactgggcag

SEQ ID NO: 236 - RNA, 21 nt, synthetic construct
  source 1..21: mol_type = other RNA
actatgacctcgaaactgggc

SEQ ID NO: 237 - RNA, 21 nt, synthetic construct
  source 1..21: mol_type = other RNA
cactatgacctcgaaactggg

SEQ ID NO: 238 - RNA, 21 nt, synthetic construct
  source 1..21: mol_type = other RNA
tccactatgacctcgaaactg

SEQ ID NO: 239 - RNA, 21 nt, synthetic construct
  source 1..21: mol_type = other RNA
aggctccactatgacctcgaa

SEQ ID NO: 240 - RNA, 21 nt, synthetic construct
  source 1..21: mol_type = other RNA
tttctctgtaggctccactat

SEQ ID NO: 241 - RNA, 21 nt, synthetic construct
  source 1..21: mol_type = other RNA
atgtagtagaatttctctgta

SEQ ID NO: 242 - RNA, 21 nt, synthetic construct
  source 1..21: mol_type = other RNA
tatagatgtagtagaatttct

SEQ ID NO: 243 - RNA, 21 nt, synthetic construct
  source 1..21: mol_type = other RNA
agatgacaaaggcagttccct

SEQ ID NO: 244 - RNA, 21 nt, synthetic construct
  source 1..21: mol_type = other RNA
aagatgacaaaggcagttccc

SEQ ID NO: 245 - RNA, 21 nt, synthetic construct
  source 1..21: mol_type = other RNA
atcccgaagatgacaaaggca

SEQ ID NO: 246 - RNA, 21 nt, synthetic construct
  source 1..21: mol_type = other RNA
atgcgcttgagggattcaggc

SEQ ID NO: 247 - RNA, 21 nt, synthetic construct
  source 1..21: mol_type = other RNA
tgcaccatgtcactgcctgag

SEQ ID NO: 248 - RNA, 21 nt, synthetic construct
  source 1..21: mol_type = other RNA
tctggtagggagaggtcacga

SEQ ID NO: 249 - RNA, 21 nt, synthetic construct
  source 1..21: mol_type = other RNA
atgaggtcaaagggcattcct

SEQ ID NO: 250 - RNA, 21 nt, synthetic construct
  source 1..21: mol_type = other RNA
aacaccatgaggtcaaagggc

SEQ ID NO: 251 - RNA, 21 nt, synthetic construct
  source 1..21: mol_type = other RNA
tcacgaacaccatgaggtcaa

SEQ ID NO: 252 - RNA, 21 nt, synthetic construct
  source 1..21: mol_type = other RNA
tcgtcacgaacaccatgaggt

SEQ ID NO: 253 - RNA, 21 nt, synthetic construct
  source 1..21: mol_type = other RNA
ttcgtcacgaacaccatgagg

SEQ ID NO: 254 - RNA, 21 nt, synthetic construct
  source 1..21: mol_type = other RNA
tgggttagagactgcacagtg

SEQ ID NO: 255 - RNA, 21 nt, synthetic construct
  source 1..21: mol_type = other RNA
atgctcaagggcttctggctg

SEQ ID NO: 256 - RNA, 21 nt, synthetic construct
  source 1..21: mol_type = other RNA
tgatgctcaagggcttctggc

SEQ ID NO: 257 - RNA, 21 nt, synthetic construct
  source 1..21: mol_type = other RNA
ttcgtgcgcaccgtgatgctc

SEQ ID NO: 258 - RNA, 21 nt, synthetic construct
  source 1..21: mol_type = other RNA
tgcttcttcgtgcgcaccgtg

SEQ ID NO: 259 - RNA, 21 nt, synthetic construct
  source 1..21: mol_type = other RNA
ttgttggagttgcccacggtg

SEQ ID NO: 260 - RNA, 21 nt, synthetic construct
  source 1..21: mol_type = other RNA
attgttggagttgcccacggt

SEQ ID NO: 261 - RNA, 21 nt, synthetic construct
  source 1..21: mol_type = other RNA
aattgttggagttgcccacgg

SEQ ID NO: 262 - RNA, 21 nt, synthetic construct
  source 1..21: mol_type = other RNA
aggtaattgttggagttgccc

SEQ ID NO: 263 - RNA, 21 nt, synthetic construct
  source 1..21: mol_type = other RNA
atgcaggtaattgttggagtt

SEQ ID NO: 264 - RNA, 21 nt, synthetic construct
  source 1..21: mol_type = other RNA
tgacgttgagggtctccccgg

SEQ ID NO: 265 - RNA, 21 nt, synthetic construct
  source 1..21: mol_type = other RNA
ttgacgttgagggtctccccg

SEQ ID NO: 266 - RNA, 21 nt, synthetic construct
  source 1..21: mol_type = other RNA
agttgacgttgagggtctccc

SEQ ID NO: 267 - RNA, 21 nt, synthetic construct
  source 1..21: mol_type = other RNA
aggaagttgacgttgagggtc

SEQ ID NO: 268 - RNA, 21 nt, synthetic construct
  source 1..21: mol_type = other RNA
attcgcaggaggaagttgacg

SEQ ID NO: 269 - RNA, 21 nt, synthetic construct
  source 1..21: mol_type = other RNA
agtagcggatcttggcctcgt

SEQ ID NO: 270 - RNA, 21 nt, synthetic construct
  source 1..21: mol_type = other RNA
taggtgtagtagcggatcttg

SEQ ID NO: 271 - RNA, 21 nt, synthetic construct
  source 1..21: mol_type = other RNA
tcaggtaggtgtagtagcgga

SEQ ID NO: 272 - RNA, 21 nt, synthetic construct
  source 1..21: mol_type = other RNA
atcaggtaggtgtagtagcgg

SEQ ID NO: 273 - RNA, 21 nt, synthetic construct
  source 1..21: mol_type = other RNA
ttgacgtccacccacacggag

SEQ ID NO: 274 - RNA, 21 nt, synthetic construct
  source 1..21: mol_type = other RNA
ttttaccaccagcgagcccac

SEQ ID NO: 275 - RNA, 21 nt, synthetic construct
  source 1..21: mol_type = other RNA
tcaccctctatcttcagggtc

SEQ ID NO: 276 - RNA, 21 nt, synthetic construct
  source 1..21: mol_type = other RNA
acctcatggggttctcccgca

SEQ ID NO: 277 - RNA, 21 nt, synthetic construct
  source 1..21: mol_type = other RNA
aacctcatggggttctcccgc

SEQ ID NO: 278 - RNA, 21 nt, synthetic construct
  source 1..21: mol_type = other RNA
agaacctcatggggttctccc

SEQ ID NO: 279 - RNA, 21 nt, synthetic construct
  source 1..21: mol_type = other RNA
tgtgatgtagttgcagcagtc

SEQ ID NO: 280 - RNA, 21 nt, synthetic construct
  source 1..21: mol_type = other RNA
tcctcatccaggttactcctg

SEQ ID NO: 281 - RNA, 21 nt, synthetic construct
  source 1..21: mol_type = other RNA
atgtcctcatccaggttactc

SEQ ID NO: 282 - RNA, 21 nt, synthetic construct
  source 1..21: mol_type = other RNA
aaacgatgttctcttctgcaa

SEQ ID NO: 283 - RNA, 21 nt, synthetic construct
  source 1..21: mol_type = other RNA
ttcgggaaacgatgttctctt

SEQ ID NO: 284 - RNA, 21 nt, synthetic construct
  source 1..21: mol_type = other RNA
tctgggaactcacttcgggaa

SEQ ID NO: 285 - RNA, 21 nt, synthetic construct
  source 1..21: mol_type = other RNA
aatatattcatgagcttcgta

SEQ ID NO: 286 - RNA, 21 nt, synthetic construct
  source 1..21: mol_type = other RNA
aaatatattcatgagcttcgt

SEQ ID NO: 287 - RNA, 21 nt, synthetic construct
  source 1..21: mol_type = other RNA
ttactgtgacctcgaaggggt

SEQ ID NO: 288 - RNA, 21 nt, synthetic construct
  source 1..21: mol_type = other RNA
attactgtgacctcgaagggg

SEQ ID NO: 289 - RNA, 21 nt, synthetic construct
  source 1..21: mol_type = other RNA
aagtcctgcattactgtgacc

SEQ ID NO: 290 - RNA, 21 nt, synthetic construct
  source 1..21: mol_type = other RNA
agagtagggtagccgcaggtc

SEQ ID NO: 291 - RNA, 21 nt, synthetic construct
  source 1..21: mol_type = other RNA
aacagagtagggtagccgcag

SEQ ID NO: 292 - RNA, 21 nt, synthetic construct
  source 1..21: mol_type = other RNA
acaacagagtagggtagccgc

SEQ ID NO: 293 - RNA, 21 nt, synthetic construct
  source 1..21: mol_type = other RNA
aacaacagagtagggtagccg

SEQ ID NO: 294 - RNA, 21 nt, synthetic construct
  source 1..21: mol_type = other RNA
tcgaacaacagagtagggtag

SEQ ID NO: 295 - RNA, 21 nt, synthetic construct
  source 1..21: mol_type = other RNA
ttcgaacaacagagtagggta

SEQ ID NO: 296 - RNA, 21 nt, synthetic construct
  source 1..21: mol_type = other RNA
tttcgaacaacagagtagggt

SEQ ID NO: 297 - RNA, 21 nt, synthetic construct
  source 1..21: mol_type = other RNA
tttccacctgctcgtttcgaa

SEQ ID NO: 298 - RNA, 21 nt, synthetic construct
  source 1..21: mol_type = other RNA
atttccacctgctcgtttcga

SEQ ID NO: 299 - RNA, 21 nt, synthetic construct
  source 1..21: mol_type = other RNA
tcggatttccacctgctcgtt

SEQ ID NO: 300 - RNA, 21 nt, synthetic construct
  source 1..21: mol_type = other RNA
ttggttctgccggtaattgta

SEQ ID NO: 301 - RNA, 21 nt, synthetic construct
  source 1..21: mol_type = other RNA
ttgtggagtagttccaccctc

SEQ ID NO: 302 - RNA, 21 nt, synthetic construct
  source 1..21: mol_type = other RNA
attgtggagtagttccaccct

SEQ ID NO: 303 - RNA, 21 nt, synthetic construct
  source 1..21: mol_type = other RNA
tggattgtggagtagttccac

SEQ ID NO: 304 - RNA, 21 nt, synthetic construct
  source 1..21: mol_type = other RNA
ttacggtctgctggtgacgcc

SEQ ID NO: 305 - RNA, 21 nt, synthetic construct
  source 1..21: mol_type = other RNA
tggttacggtctgctggtgac

SEQ ID NO: 306 - RNA, 21 nt, synthetic construct
  source 1..21: mol_type = other RNA
acgaccttcagggacttcctg

SEQ ID NO: 307 - RNA, 21 nt, synthetic construct
  source 1..21: mol_type = other RNA
tgattccttccggcacgacct

SEQ ID NO: 308 - RNA, 21 nt, synthetic construct
  source 1..21: mol_type = other RNA
tctgattccttccggcacgac

SEQ ID NO: 309 - RNA, 21 nt, synthetic construct
  source 1..21: mol_type = other RNA
ttctgattccttccggcacga

SEQ ID NO: 310 - RNA, 21 nt, synthetic construct
  source 1..21: mol_type = other RNA
tcattctgattccttccggca

SEQ ID NO: 311 - RNA, 21 nt, synthetic construct
  source 1..21: mol_type = other RNA
ttcattctgattccttccggc

SEQ ID NO: 312 - RNA, 21 nt, synthetic construct
  source 1..21: mol_type = other RNA
ttggtcactgaggtctgcagg

SEQ ID NO: 313 - RNA, 21 nt, synthetic construct
  source 1..21: mol_type = other RNA
ttgcaggagaattctggtctc

SEQ ID NO: 314 - RNA, 21 nt, synthetic construct
  source 1..21: mol_type = other RNA
tgaggtgcttcagccgttccg

SEQ ID NO: 315 - RNA, 21 nt, synthetic construct
  source 1..21: mol_type = other RNA
atccaggtaatgcacagcgat

SEQ ID NO: 316 - RNA, 21 nt, synthetic construct
  source 1..21: mol_type = other RNA
cgtttcatccaggtaatgcac

SEQ ID NO: 317 - RNA, 21 nt, synthetic construct
  source 1..21: mol_type = other RNA
ttcttgatgagctccaaggcc

SEQ ID NO: 318 - RNA, 21 nt, synthetic construct
  source 1..21: mol_type = other RNA
ttgtctgaaggccagctgctg

SEQ ID NO: 319 - RNA, 21 nt, synthetic construct
  source 1..21: mol_type = other RNA
accttgaccacgtaggcggtc

SEQ ID NO: 320 - RNA, 21 nt, synthetic construct
  source 1..21: mol_type = other RNA
aagaccttgaccacgtaggcg

SEQ ID NO: 321 - RNA, 21 nt, synthetic construct
  source 1..21: mol_type = other RNA
agagaagaccttgaccacgta

SEQ ID NO: 322 - RNA, 21 nt, synthetic construct
  source 1..21: mol_type = other RNA
atgaggttgacagccagagag

SEQ ID NO: 323 - RNA, 21 nt, synthetic construct
  source 1..21: mol_type = other RNA
atttaacagccccgcagagga

SEQ ID NO: 324 - RNA, 21 nt, synthetic construct
  source 1..21: mol_type = other RNA
aggatcagccatttaacagcc

SEQ ID NO: 325 - RNA, 21 nt, synthetic construct
  source 1..21: mol_type = other RNA
tatcacgggcgcatcctcctg

SEQ ID NO: 326 - RNA, 21 nt, synthetic construct
  source 1..21: mol_type = other RNA
aacaaaggccgtgagggccat

SEQ ID NO: 327 - RNA, 21 nt, synthetic construct
  source 1..21: mol_type = other RNA
tgagaacaaaggccgtgaggg

SEQ ID NO: 328 - RNA, 21 nt, synthetic construct
  source 1..21: mol_type = other RNA
agcgagatgagaacaaaggcc

SEQ ID NO: 329 - RNA, 21 nt, synthetic construct
  source 1..21: mol_type = other RNA
tcatgtagttggcttcaagga

SEQ ID NO: 330 - RNA, 21 nt, synthetic construct
  source 1..21: mol_type = other RNA
tgtaggttcatgtagttggct

SEQ ID NO: 331 - RNA, 21 nt, synthetic construct
  source 1..21: mol_type = other RNA
agtgtaggatctctgtaggtt

SEQ ID NO: 332 - RNA, 21 nt, synthetic construct
  source 1..21: mol_type = other RNA
tatctttggctgtggtcagaa

SEQ ID NO: 333 - RNA, 21 nt, synthetic construct
  source 1..21: mol_type = other RNA
ttcttatctttggctgtggtc

SEQ ID NO: 334 - RNA, 21 nt, synthetic construct
  source 1..21: mol_type = other RNA
agcggttcttatctttggctg

SEQ ID NO: 335 - RNA, 21 nt, synthetic construct
  source 1..21: mol_type = other RNA
agagggcataggatgtggcct

SEQ ID NO: 336 - RNA, 21 nt, synthetic construct
  source 1..21: mol_type = other RNA
aagagggcataggatgtggcc

SEQ ID NO: 337 - RNA, 21 nt, synthetic construct
  source 1..21: mol_type = other RNA
ttttagctgcagtagggccaa

SEQ ID NO: 338 - RNA, 21 nt, synthetic construct
  source 1..21: mol_type = other RNA
agtcttttagctgcagtaggg

SEQ ID NO: 339 - RNA, 21 nt, synthetic construct
  source 1..21: mol_type = other RNA
agtcaaagtcttttagctgca

SEQ ID NO: 340 - RNA, 21 nt, synthetic construct
  source 1..21: mol_type = other RNA
aaagtcaaagtcttttagctg

SEQ ID NO: 341 - RNA, 21 nt, synthetic construct
  source 1..21: mol_type = other RNA
ttgagccaacgcacgacggga

SEQ ID NO: 342 - RNA, 21 nt, synthetic construct
  source 1..21: mol_type = other RNA
attgagccaacgcacgacggg

SEQ ID NO: 343 - RNA, 21 nt, synthetic construct
  source 1..21: mol_type = other RNA
ttcattgagccaacgcacgac

SEQ ID NO: 344 - RNA, 21 nt, synthetic construct
  source 1..21: mol_type = other RNA
tctgttcattgagccaacgca

SEQ ID NO: 345 - RNA, 21 nt, synthetic construct
  source 1..21: mol_type = other RNA
tatctctgttcattgagccaa

SEQ ID NO: 346 - RNA, 21 nt, synthetic construct
  source 1..21: mol_type = other RNA
agtatctctgttcattgagcc

SEQ ID NO: 347 - RNA, 21 nt, synthetic construct
  source 1..21: mol_type = other RNA
tggaacaccatgaaggtggcc

SEQ ID NO: 348 - RNA, 21 nt, synthetic construct
  source 1..21: mol_type = other RNA
ttggaacaccatgaaggtggc

SEQ ID NO: 349 - RNA, 21 nt, synthetic construct
  source 1..21: mol_type = other RNA
agccaaggcttggaacaccat

SEQ ID NO: 350 - RNA, 21 nt, synthetic construct
  source 1..21: mol_type = other RNA
agattcccagtggatacggtg

SEQ ID NO: 351 - RNA, 21 nt, synthetic construct
  source 1..21: mol_type = other RNA
tcttctgatcgcaggaggctg

SEQ ID NO: 352 - RNA, 21 nt, synthetic construct
  source 1..21: mol_type = other RNA
ttggtctcttctgatcgcagg

SEQ ID NO: 353 - RNA, 21 nt, synthetic construct
  source 1..21: mol_type = other RNA
tccttggtctcttctgatcgc

SEQ ID NO: 354 - RNA, 21 nt, synthetic construct
  source 1..21: mol_type = other RNA
tcagctgtgactgtgaaaccc

SEQ ID NO: 355 - RNA, 21 nt, synthetic construct
  source 1..21: mol_type = other RNA
ttagcatggtacattgtcacc

SEQ ID NO: 356 - RNA, 21 nt, synthetic construct
  source 1..21: mol_type = other RNA
tttggccttagcatggtacat

SEQ ID NO: 357 - RNA, 21 nt, synthetic construct
  source 1..21: mol_type = other RNA
atttattacaggtgagttgat

SEQ ID NO: 358 - RNA, 21 nt, synthetic construct
  source 1..21: mol_type = other RNA
aggtcgaatttattacaggtg

SEQ ID NO: 359 - RNA, 21 nt, synthetic construct
  source 1..21: mol_type = other RNA
ttgaggtcgaatttattacag

SEQ ID NO: 360 - RNA, 21 nt, synthetic construct
  source 1..21: mol_type = other RNA
tatggtgaccttgaggtcgaa

SEQ ID NO: 361 - RNA, 21 nt, synthetic construct
  source 1..21: mol_type = other RNA
ttatggtgaccttgaggtcga

SEQ ID NO: 362 - RNA, 21 nt, synthetic construct
  source 1..21: mol_type = other RNA
tggttttatggtgaccttgag

SEQ ID NO: 363 - RNA, 21 nt, synthetic construct
  source 1..21: mol_type = other RNA
tttctgtttccggtgctggtt

SEQ ID NO: 364 - RNA, 21 nt, synthetic construct
  source 1..21: mol_type = other RNA
tcttttctgtttccggtgctg

SEQ ID NO: 365 - RNA, 21 nt, synthetic construct
  source 1..21: mol_type = other RNA
ttcttggcatcctgaggcctc

SEQ ID NO: 366 - RNA, 21 nt, synthetic construct
  source 1..21: mol_type = other RNA
tagtgttcttggcatcctgag

SEQ ID NO: 367 - RNA, 21 nt, synthetic construct
  source 1..21: mol_type = other RNA
tcatagtgttcttggcatcct

SEQ ID NO: 368 - RNA, 21 nt, synthetic construct
  source 1..21: mol_type = other RNA
aggatcatagtgttcttggca

SEQ ID NO: 369 - RNA, 21 nt, synthetic construct
  source 1..21: mol_type = other RNA
tcaaggatcatagtgttcttg

SEQ ID NO: 370 - RNA, 21 nt, synthetic construct
  source 1..21: mol_type = other RNA
atagtggcatcctggtctccc

SEQ ID NO: 371 - RNA, 21 nt, synthetic construct
  source 1..21: mol_type = other RNA
agacatagtggcatcctggtc

SEQ ID NO: 372 - RNA, 21 nt, synthetic construct
  source 1..21: mol_type = other RNA
tagacatagtggcatcctggt

SEQ ID NO: 373 - RNA, 21 nt, synthetic construct
  source 1..21: mol_type = other RNA
tatagacatagtggcatcctg

SEQ ID NO: 374 - RNA, 21 nt, synthetic construct
  source 1..21: mol_type = other RNA
atatagacatagtggcatcct

SEQ ID NO: 375 - RNA, 21 nt, synthetic construct
  source 1..21: mol_type = other RNA
tggagatgtatctgtcaacac

SEQ ID NO: 376 - RNA, 21 nt, synthetic construct
  source 1..21: mol_type = other RNA
acttggagatgtatctgtcaa

SEQ ID NO: 377 - RNA, 21 nt, synthetic construct
  source 1..21: mol_type = other RNA
atacttggagatgtatctgtc

SEQ ID NO: 378 - RNA, 21 nt, synthetic construct
  source 1..21: mol_type = other RNA
catacttggagatgtatctgt

SEQ ID NO: 379 - RNA, 21 nt, synthetic construct
  source 1..21: mol_type = other RNA
tcatacttggagatgtatctg

SEQ ID NO: 380 - RNA, 21 nt, synthetic construct
  source 1..21: mol_type = other RNA
ttgtccagctcatacttggag

SEQ ID NO: 381 - RNA, 21 nt, synthetic construct
  source 1..21: mol_type = other RNA
atcggagaaggctttgtccag

SEQ ID NO: 382 - RNA, 21 nt, synthetic construct
  source 1..21: mol_type = other RNA
tatcggagaaggctttgtcca

SEQ ID NO: 383 - RNA, 21 nt, synthetic construct
  source 1..21: mol_type = other RNA
tgttcctatcggagaaggctt

SEQ ID NO: 384 - RNA, 21 nt, synthetic construct
  source 1..21: mol_type = other RNA
atgagggtgttcctatcggag

SEQ ID NO: 385 - RNA, 21 nt, synthetic construct
  source 1..21: mol_type = other RNA
tgatgagggtgttcctatcgg

SEQ ID NO: 386 - RNA, 21 nt, synthetic construct
  source 1..21: mol_type = other RNA
agtgtgagaccttgtccaggt

SEQ ID NO: 387 - RNA, 21 nt, synthetic construct
  source 1..21: mol_type = other RNA
attggtgaactttgaaagcta

SEQ ID NO: 388 - RNA, 21 nt, synthetic construct
  source 1..21: mol_type = other RNA
tattggtgaactttgaaagct

SEQ ID NO: 389 - RNA, 21 nt, synthetic construct
  source 1..21: mol_type = other RNA
taggcgtagaccttgactgct

SEQ ID NO: 390 - RNA, 21 nt, synthetic construct
  source 1..21: mol_type = other RNA
aataggcgtagaccttgactg

SEQ ID NO: 391 - RNA, 21 nt, synthetic construct
  source 1..21: mol_type = other RNA
ttgtaataggcgtagaccttg

SEQ ID NO: 392 - RNA, 21 nt, synthetic construct
  source 1..21: mol_type = other RNA
tggtagaaccgggtacagctt

SEQ ID NO: 393 - RNA, 21 nt, synthetic construct
  source 1..21: mol_type = other RNA
atggtagaaccgggtacagct

SEQ ID NO: 394 - RNA, 21 nt, synthetic construct
  source 1..21: mol_type = other RNA
ttccatcctccttttccggat

SEQ ID NO: 395 - RNA, 21 nt, synthetic construct
  source 1..21: mol_type = other RNA
tttccatcctccttttccgga

SEQ ID NO: 396 - RNA, 21 nt, synthetic construct
  source 1..21: mol_type = other RNA
tgttcagctttccatcctcct

SEQ ID NO: 397 - RNA, 21 nt, synthetic construct
  source 1..21: mol_type = other RNA
ttctcctcagcacagcggcac

SEQ ID NO: 398 - RNA, 21 nt, synthetic construct
  source 1..21: mol_type = other RNA
attctcctcagcacagcggca

SEQ ID NO: 399 - RNA, 21 nt, synthetic construct
  source 1..21: mol_type = other RNA
aattctcctcagcacagcggc

SEQ ID NO: 400 - RNA, 21 nt, synthetic construct
  source 1..21: mol_type = other RNA
aagcaattctcctcagcacag

SEQ ID NO: 401 - RNA, 21 nt, synthetic construct
  source 1..21: mol_type = other RNA
tgaagcaattctcctcagcac

SEQ ID NO: 402 - RNA, 21 nt, synthetic construct
  source 1..21: mol_type = other RNA
ttgtatgaagcaattctcctc

SEQ ID NO: 403 - RNA, 21 nt, synthetic construct
  source 1..21: mol_type = other RNA
tttgtatgaagcaattctcct

SEQ ID NO: 404 - RNA, 21 nt, synthetic construct
  source 1..21: mol_type = other RNA
tagtccactcctggctcacag

SEQ ID NO: 405 - RNA, 21 nt, synthetic construct
  source 1..21: mol_type = other RNA
acacatagtccactcctggct

SEQ ID NO: 406 - RNA, 21 nt, synthetic construct
  source 1..21: mol_type = other RNA
tacacatagtccactcctggc

SEQ ID NO: 407 - RNA, 21 nt, synthetic construct
  source 1..21: mol_type = other RNA
tgtacacatagtccactcctg

SEQ ID NO: 408 - RNA, 21 nt, synthetic construct
  source 1..21: mol_type = other RNA
ttgtacacatagtccactcct

SEQ ID NO: 409 - RNA, 21 nt, synthetic construct
  source 1..21: mol_type = other RNA
tcttgtacacatagtccactc

SEQ ID NO: 410 - RNA, 21 nt, synthetic construct
  source 1..21: mol_type = other RNA
tactcgtcaaagtcattggac

SEQ ID NO: 411 - RNA, 21 nt, synthetic construct
  source 1..21: mol_type = other RNA
tgatgtactcgtcaaagtcat

SEQ ID NO: 412 - RNA, 21 nt, synthetic construct
  source 1..21: mol_type = other RNA
atgatgtactcgtcaaagtca

SEQ ID NO: 413 - RNA, 21 nt, synthetic construct
  source 1..21: mol_type = other RNA
tggccatgatgtactcgtcaa

SEQ ID NO: 414 - RNA, 21 nt, synthetic construct
  source 1..21: mol_type = other RNA
atccgagcctgacttgatggt

SEQ ID NO: 415 - RNA, 21 nt, synthetic construct
  source 1..21: mol_type = other RNA
tgcacctcatccgagcctgac

SEQ ID NO: 416 - RNA, 21 nt, synthetic construct
  source 1..21: mol_type = other RNA
acctgcacctcatccgagcct

SEQ ID NO: 417 - RNA, 21 nt, synthetic construct
  source 1..21: mol_type = other RNA
ttgatggggctgatgaacgtg

SEQ ID NO: 418 - RNA, 21 nt, synthetic construct
  source 1..21: mol_type = other RNA
aaatcggaggagagaccccac

SEQ ID NO: 419 - RNA, 21 nt, synthetic construct
  source 1..21: mol_type = other RNA
ttctctccccagaaatcggag

SEQ ID NO: 420 - RNA, 21 nt, synthetic construct
  source 1..21: mol_type = other RNA
tcccgatgatgtagctgaggt

SEQ ID NO: 421 - RNA, 21 nt, synthetic construct
  source 1..21: mol_type = other RNA
tccttcccgatgatgtagctg

SEQ ID NO: 422 - RNA, 21 nt, synthetic construct
  source 1..21: mol_type = other RNA
tggcattcgtcctcctcgggc

SEQ ID NO: 423 - RNA, 21 nt, synthetic construct
  source 1..21: mol_type = other RNA
ttggcattcgtcctcctcggg

SEQ ID NO: 424 - RNA, 21 nt, synthetic construct
  source 1..21: mol_type = other RNA
tcagttggggcacccaaagac